European Patent Application EP 4 620 967 A1, published September 24, 2025. Title: Peptide having activities of skin condition improvement and uses thereof. Applicant: CAREGEN CO., LTD. The sequence listing filed with the application follows.

SEQUENCE LISTING (13 sequences)

SEQ ID NO: 1 - protein, 8 aa, synthetic construct
TNRTEVEG

SEQ ID NO: 2 - DNA, 20 bp, synthetic construct
  source 1..20: mol_type = other DNA
caccctcaagagcctgagtc

SEQ ID NO: 3 - DNA, 20 bp, synthetic construct
  source 1..20: mol_type = other DNA
agacggctgagtagggaaca

SEQ ID NO: 4 - DNA, 20 bp, synthetic construct
  source 1..20: mol_type = other DNA
ccaggaaccgagtacaccat

SEQ ID NO: 5 - DNA, 20 bp, synthetic construct
  source 1..20: mol_type = other DNA
atacccaggttgggtgatga

SEQ ID NO: 6 - DNA, 20 bp, synthetic construct
  source 1..20: mol_type = other DNA
gcaagacctggctttggact

SEQ ID NO: 7 - DNA, 21 bp, synthetic construct
  source 1..21: mol_type = other DNA
gggagtttctggttagggctg

SEQ ID NO: 8 - DNA, 20 bp, synthetic construct
  source 1..20: mol_type = other DNA
ggagccaaaagggtcatcat

SEQ ID NO: 9 - DNA, 20 bp, synthetic construct
  source 1..20: mol_type = other DNA
gtgatggcatggactgtggt

SEQ ID NO: 10 - DNA, 20 bp, synthetic construct
  source 1..20: mol_type = other DNA
tcagtggctggaacagtgag

SEQ ID NO: 11 - DNA, 20 bp, synthetic construct
  source 1..20: mol_type = other DNA
tctggcatgtcccactatca

SEQ ID NO: 12 - DNA, 20 bp, synthetic construct
  source 1..20: mol_type = other DNA
ccttcttgggtgctggaata

SEQ ID NO: 13 - DNA, 20 bp, synthetic construct
  source 1..20: mol_type = other DNA
acacgataagggaggctgtg